European Patent Specification EP 3 554 503 B1, published October 4, 2023. Title: INHIBITORS OF BROMODOMAIN-CONTAINING PROTEIN 4 (BRD4). Applicant: ZHOU, Jia BRASIER, Allan R. TIAN, Bing LIU, Zhiqing CHEN, Haiying RYTTING, Erik. Application PCT/US2017/066107. The sequence listing filed with the application follows.

SEQUENCE LISTING (2 sequences)

SEQ ID NO: 1 - DNA, 25 bp, Artificial Sequence
  Synthetic Primer
tgcaaacagacctcctttgtcttga

SEQ ID NO: 2 - DNA, 23 bp, Artificial Sequence
  Synthetic Primer
tcctgagaccagactcctcctcc